European Patent Application EP 4 458 972 A1, published November 6, 2024. Title: USE OF ASPARTATE DECARBOXYLASE IN FERMENTATION PRODUCTION OF VITAMIN B5. Applicant: 中国科学院微生物研究所. Application CN. The sequence listing filed with the application follows.

SEQUENCE LISTING (49 sequences)

SEQ ID NO: 1 - DNA, 372 bp, (Artificial Sequence)
  source 1..372: mol_type = genomic DNA
atgatggccggaaaactgcaccgcgctaccgtgacggaagccaatttaaactatgtcggcagcataacgattgatgaagatcttttagatgccgtcggaatgctcgctaatgaaaaagttcagattgtgaataataataacggagcgagacttgaaacgtatattattcccggtaagcgggggagcggcgtcatctgtttaaatggagctgccgcccgtctcgtccaagaaggagataaagtcattattatttcttatcaaatgatgtctgatcaggaagcaaaaagccatcagccgaaggtggccgttctggatgatcagaataaaatcgagcagatgctgggccaggagccggcacacacgattttgtaa

SEQ ID NO: 2 - DNA, 384 bp, (Artificial Sequence)
  source 1..384: mol_type = genomic DNA
atgtatcgaacaatgatgagcggcaaacttcacagggcaactgttacggaagcaaacctgaactatgtgggaagcattacaattgatgaagatctcattgatgctgtgggaatgcttcctaatgaaaaagtacaaattgtgaataataataatggagcacgtcttgaaacgtatattattcctggtaaacggggaagcggcgtcatatgcttaaacggtgcagccgcacgccttgtgcaggaaggagataaggtcattattatttcctacaaaatgatgtctgatcaagaagcggcaagccatgagccgaaagtggctgttctgaatgatcaaaacaaaattgaacaaatgctggggaacgaaccagcccgtacaattttgtaa

SEQ ID NO: 3 - DNA, 384 bp, (Artificial Sequence)
  source 1..384: mol_type = genomic DNA
atgtaccgtacgttaatgagcgcaaaacttcacagagcgagagtgacggaagccaatttgaactacgtcggcagcgtgacaattgatgaagatttgctggatgctgtcggaatgatggcaaatgaaaaagtgcaaattgtgaataataataacggggcccggctggaaacgtacattattcccggtgaaaggggcagcggcgtcgtttgtttaaacggagctgccgcccgccttgtccaggttggagatgtcgtcatcatcgtgtcttatgcgatgatgtctgaagaggaagcaaagacccataagccgaaggttgccgttttgaacgagagaaacgaaatcgaggaaatgctgggtcaggagccagcccgtaccattctgtaa

SEQ ID NO: 4 - DNA, 396 bp, (Artificial Sequence)
  source 1..396: mol_type = genomic DNA
atgaagctgcacctgctgaagagcaaaattcacaacgcgcgtgttaccagcggtgacctggagtacgaaggcagcattaccatcgatcaggagctgctgctgctggcggagatgatcccgaacgaaaaagttctggtggtgaacaacaacaacggcgagcgtttcgaaacctatatcattaacggtgaaccgggcagccgtgttattcagctgaacggtgcggcggcgcgttgcgcgctgccgggcgacgagatcattatcatgaccttcgcggtgatggatgaaaagaaagcgcgtacctttcaaccgatggtgctgatcgttgaccacctgaacaacccgaagcgtcgtcaccgtattggccaggaagacgaacaactgagcagcagcatctaa

SEQ ID NO: 5 - DNA, 411 bp, (Artificial Sequence)
  source 1..411: mol_type = genomic DNA
atgctgcgcaccatcctcggtagcaagattcaccgcgccaccgtcacccaggccgaccttgactatgtcggctccatcaccatcgacgccgacctggtcaatgccgccggcctcatcgagggcgagaaggtcgccgtcgtggacatcaccaacggcgcccgcattgagacctatgtgatcaccggcgatgccggaaccggcagcatctgcatcaatggtgccgccgcccatctgatcaacccgggtgatctggtcatcatcatgagctatctgcaggccaccgatgccgaggcccgcgcctaccagcccaatatcgtccacgtggatgccgacaaccggatcgtcgccctgggcaacgacgccggcgagcccatcccgggttccagcttgctgtcctcgcgctccctctaa

SEQ ID NO: 6 - DNA, 411 bp, (Artificial Sequence)
  source 1..411: mol_type = genomic DNA
atgctgcgcaccatcctcggaagtaagattcaccgagccactgtcactcaagctgatctagattatgttggctctgtaaccatcgacgccgacctggttcacgccgccggattgatcgaaggcgaaaaagttgccatcgtagacatcaccaacggcgctcgtctggaaacttatgtcattgtgggcgacgccggaacgggcaatatttgcatcaatggtgccgctgcacaccttattaatcctggcgatcttgtgatcatcatgagctaccttcaggcaactgatgcggaagccaaggcgtatgagccaaagattgtgcacgtggacgccgacaaccgcatcgttgcgctcggcaacgatcttgcggaagcactacctggatccgggcttttgacgtcgagaagcatttaa

SEQ ID NO: 7 - DNA, 411 bp, (Artificial Sequence)
  source 1..411: mol_type = genomic DNA
atgctcagaaccatcctcggcagcaaaatccaccgcgccacggtcacccaggcagacctcaactacgtggggtccgtcacggtcgacgccgacctgctcgcggccgccggcctcatcgagggcgaaaaggtggccatcgtcgacgtcaccaacggtgccaggctggagacctacgtcatcaccggtcgcccgggcaccggcgagatctgcatcaacggtgcggcggcgcacctgatccacccgggcgacatcgtcatcctcatctcctacctgcaggccaccctggacgaggccctcgaatacgagccgcgcatcgtccacgtcgacgagaacaaccgcatcgtcgccctgggcaatgacatcgccgaggccgtcccgggctccgacaccgtctccgcccggaacatctaa

SEQ ID NO: 8 - DNA, 381 bp, (Artificial Sequence)
  source 1..381: mol_type = genomic DNA
atgattcgcacgatgctgcagggcaaactccaccgcgtgaaagtgactcatgcggacctgcactatgaaggttcttgcgccattgaccaggattttcttgacgcagccggtattctcgaaaacgaagccattgatatctggaatgtcaccaacggcaagcgtttctccacttatgccatcgcggcagaacgcggttcgagaattatttctgttaacggtgcggcggcccactgcgccagtgtcggcgatattgtcatcatcgccagcttcgttaccatgccagatgaagaagctcgcacctggcgacccaacgtcgcctattttgaaggcgacaatgaaatgaaacgtaccgcgaaagcgattccggtacaggttgcttaa

SEQ ID NO: 9 - DNA, 345 bp, (Artificial Sequence)
  source 1..345: mol_type = genomic DNA
atgcgtcgttggctgctgaagagcaaactgcaccgtgcgcgtgtgaccggtaccgagaaggactacgaaggcagcatcagcattgatgcggcgctgctgagcgaggcggacattgcggtgggtgaacaggttcaagtggttaacgttaccaacggcgagcgtttcgaaacctataccattgagggtgaaagccgtcagatggagctgaacggtgcggcggcgcgtctggcggaaaccggtgatgtgatcattgttatcagctacggcctgtatgtgaaagatgagcaaccggaaccgaccgttctgctgctggacgaggaaaaccgtattagcgagcgtgaataa

SEQ ID NO: 10 - DNA, 228 bp, (Artificial Sequence)
  source 1..228: mol_type = genomic DNA
atgcagcgtaccttcctgaagagcaaactgcaccgtctgaccaccaccatccgtggcaaggagaacagcggcgtgattctggttaacggtgtggcgccgcacaaagttgcgggcgacctgctgatcattgcggcgtacagcagctatagcgaggatgaactgcgtaactaccaaccggcgctgtgctatgttgacgaaaagaacgtgctgacccgtatcagccgttaa

SEQ ID NO: 11 - DNA, 1191 bp, (Artificial Sequence)
  source 1..1191: mol_type = genomic DNA
atgcgtaacatgcaggagaaaggcgtgagcgagaaggaaattctggaggaactgaagaaataccgtagcctggatctgaaatatgaagacggcaacattttcggtagcatgtgcagcaacgtgctgccgatcacccgtaagatcgttgatattttcctggagaccaacctgggtgacccgggcctgtttaaaggtaccaagctgctggaggaaaaagcggtggcgctgctgggcagcctgctgaacaacaaggatgcgtacggtcacatcgttagcggtggcaccgaagcgaacctgatggcgctgcgttgcatcaaaaacatttggcgtgagaaacgtcgtaagggcctgagcaaaaacgaacacccgaagatcattgtgccgattaccgcgcacttcagctttgagaaaggtcgtgaaatgatggatctggagtacatctatgcgccgattaaagaggactacaccatcgacgaaaaatttgtgaaggacgcggttgaggactatgatgttgacggtatcattggcattgcgggtaccaccgaactgggtaccatcgataacattgaggaactgagcaaaatcgcgaaggaaaacaacatctacattcacgtggacgcggcgttcggtggcctggttatcccgtttctggacgataaatacaagaaaaagggcgtgaactataagttcgattttagcctgggtgttgatagcatcaccattgacccgcacaaaatgggtcactgcccgatcccgagcggtggcattctgttcaaagacatcggttacaagcgttatctggatgtggacgcgccgtatctgaccgagacccgtcaggcgaccattctgggcacccgtgtgggttttggtggcgcgtgcacctacgcggttctgcgttatctgggccgtgaaggtcaacgtaaaatcgttaacgagtgcatggaaaacaccctgtacctgtataaaaagctgaaagagaacaacttcaagccggtgatcgaaccgattctgaacatcgttgcgattgaggatgaagactacaaagaggtgtgcaaaaagctgcgtgaccgtggtatttatgtgagcgtttgcaactgcgttaaagcgctgcgtatcgtggttatgccgcacattaagcgtgagcacatcgataactttatcgaaattctgaacagcatcaaacgtgactaa

SEQ ID NO: 12 - DNA, 543 bp, (Artificial Sequence)
  source 1..543: mol_type = genomic DNA
atgatgaagatcattcgtgcgaaactgcacggcatccgtgtgaccaacgcggatctgaactaccacggcagcattaccctggacccggagcagtgcgaaatggcgggtatctatccgatggagttcgttgatatttggaacaagaacagcgcggcgcgtatcagcacctacgtgatttttggtgaaccgggcagccgttgctgcgttctgaacggtgcggcggcgcgtacctgccaaaaaggcgacgagctgatcattgcggcgagcgcggatatcagcggtccggaaaagctgtacgacatcaaaccgcgtattctgaccttcctgccggacaaccacgtggatcaggttctgtactatgatgtgttccaaagcgagaagcgtccgtatgactttcgtatcgttgacgcggataaacacaccattgaaagctgccacacctggccgaacgtggacatcaccaagctgcgtagcgatctggcggcgaaaggttggagcgaggcggaaatcgacagcttcattgcgagccactttagcctgtaa

SEQ ID NO: 13 - DNA, 1506 bp, (Artificial Sequence)
  source 1..1506: mol_type = genomic DNA
atgcgtgacaccaagaaaatgctgaaccgtgcggatgagctggacgatctgtacgaagcggttcgtgcgctgatcattccgcatgtgcgtgcggcggatgaagcgtgcagcctgaagagcgcgggtcagctgcacaccgacgatacccagcgtctgcaaaacgttctggtggaaccgtacccgccgaaggcgctgcaggagcgtttccaatttaccctgccggacaacgagggtaacggcaaagatggcctgatgcacctgatccgtgatgttctgcgttatagcgtgaacacctgggaccaaggttttatggataagctgaccagcagcaccaacccggttggcgtgatcagcgaaattgttctgggcatcctgaacaccaacgttcatgtgtaccatgtggcgccggcgctgagcgttattgagaaagtgaccggccgtaccctggcggcgtatttcggttttaacagcccgagcgcgggtggcattagctgccagggtggcagcgcgagcaacctgaccagcctggtggttgcgcgtaacagcctgtacccggactgcaagctgaacggtggcagcagctatcaatttgcgatcttcaccagctgccacggtcacttcagcatggaaaaagcggcgattacctgcggtatgggcctgagcagcgtggttcacgttccggtgaacgacgatggccgtatgaacgttagcgcgctgcgtgagctggtgatccaggcgaaggcgcaaggtaaaaccccgctgtatgttaacgcgaccgcgggtaccaccgttctgggtgtgtttgacccgctgcacgaaatcaagaccatttgcgaggaatttggcatgtggttccacgtggatgcgagctggggtggcagcatcattttcagcgcgaagcaccgtcacaaactgaccggttgcgagctggcggacagcctgaccattagcccgcacaaaatgctgaacgttccgatgacctgcagctttctgctgaccaacaacctgagcagcttctacaccgcgaacagcctggacgcgggttacctgttccacgataccgaggacgatgaagtgtgggacctggcgaacctgaccctgcagtgcggtcgtcgtgcggatagcctgaaaatggcgctggcgtggacctactatggtgcggcgggctttgaacgtcgtatcaaccacgcgttcaagatggcggcgcacctgagcagcatcattcagaaaagcccggactttgaactggttagcccgaacccgccgccgtgcctgcaagtgtgcttctactataccccgggtggcaagatggcgaaaagcgagatggaaaccagccgtcgtacccgtgcgatggttgaaaagatggtggaccgtggcttcatgtttgatttcgcgccgggtccgaaaggcgatttctttcgtgtggttgtgaactgcgagaccctgctgggtaccgttgaaggcctgttcaagggtctggaggcggtgggtaaacaagttgtgtaa

SEQ ID NO: 14 - DNA, 222 bp, (Artificial Sequence)
  source 1..222: mol_type = genomic DNA
atgctgaacatcaccaccggtgcgcgtttcaccacctacgcgatcgaagcgccgcgtggcagcaaagtgattggtgtgaacggtgcggcggcgcgtctggtgcagaagggtgacaaagttatcgtggttacctacggcatgctgccggaggaagaggcgcgtaactataacccgaccgtggttctgctggacgatggtaacctgattaaacgtgcggcgtaa

SEQ ID NO: 15 - DNA, 471 bp, (Artificial Sequence)
  source 1..471: mol_type = genomic DNA
atggtggacaccccgtaccgtaagatgctggcggcgaaaatccaccgtgcgaccgtgaccggtgcggatgttaactatgaaggcagcctgaccgtgccgccggaactgctggttgcggcgaagatccacccgtacgagagcctgcacgtgtggaacgttacccgtggtacccgtctggagacctatgcgattgaaggcctgccgaacagcaacgacgtgtgcgcgaacggtgcggcggcgcacctgattcgtccgggtgaccatgtgattctggcggcgtatgcgatggttccggaggcggatgcggcgacccacaaaccgcgtctgatcttcgtggacgataacaaccagctgagccacgttggtccggaaattgcgggtccgaacctgcgtagcgacagcgacgatacccacctggttcgtagcaccgagatgaccccggatggtcaaccgctggcggaaggctgctaa

SEQ ID NO: 16 - DNA, 345 bp, (Artificial Sequence)
  source 1..345: mol_type = genomic DNA
atgctgaacatctacctgaagagcaaaatccacatggcgaccattacccgtaaagaggtgtactatgaaggtagcatcgagattgacgaggaactgatgggtaaagcgggcattagcgagggcgaactggttctggtggtgaacgttaacaacgcggaacgtttcgtgacctacgttatcaagggtaaacgtggcagccgtgagattaacctgtatggtgcggcggcgcgtctgggcgaggaaggcgaccgtgtgatcattatggcgttcacctttagcgataagccggtgaaggcgaaaaccatcgttctgaacgagaagaacgaaattgttcaggaaaaataa

SEQ ID NO: 17 - DNA, 84 bp, (Artificial Sequence)
  source 1..84: mol_type = genomic DNA
ccaagttcacttaaaaaggagatcaacaatgaaagcaattttcgtactgaaacatcttaatcatgctaaggaggttttctaatg

SEQ ID NO: 18 - DNA, 1800 bp, (Artificial Sequence)
  source 1..1800: mol_type = genomic DNA
cgcggatccttgacaattaatcatccggctcgtataatgtgtggagcacaacatcaatttatcaggatacgttatgaaaccgaccaccatctccttactgcagaagtacaaacaggaaaaaaaacgtttcgcgaccatcaccgcttatgactatagcttcgccaaactctttgctgatgaagggcttaacgtcatgctggtgggcgattcgctgggcatgacggttcaggggcacgactccaccctgccagttaccgttgccgatatcgcctaccacactgccgccgtacgtcgcggcgcaccaaactgcctgctgctggctgacctgccgtttatggcgtatgccacgccggaacaagccttcgaaaacgccgcaacggttatgcgtgccggtgctaacatggtcaaaattgaaggcggtgagtggctggtagaaaccgtacaaatgctgaccgaacgtgccgttcctgtatgtggtcacttaggtttaacaccacagtcagtgaatattttcggtggctacaaagttcaggggcgcggcgatgaagcgggcgatcaactgctcagcgatgcattagccttagaagctgctggggcacagctgctggtgctggaatgcgtgccggttgaactggcaaaacgtattaccgaagcactggcgatcccggttattggcattggcgcaggcaacgtcactgacgggcagatcctcgtgatgcacgacgcctttggtattaccggcggtcacattcctaaattcgctaaaaatttcctcgccgaaacgggcgacatccgcgcggctgtgcggcagtatatggctgaagtggagtccggcgtttatccgggcgaagaacacagtttccattaaggagtcacgttgtgttaattatcgaaaccctgccgctgctgcgtcagcaaattcgccgcctgcgtatggaaggcaagcgcgtggcgctggtgcctaccatgggtaacctgcacgatggccatatgaagctggtcgacgaagccaaagcccgcgccgatgtggtcgtcgtcagtattttcgttaacccgatgcagttcgaccgcccggaagatctggctcgttatccacggaccttgcaggaggactgcgagaagctaaacaaacgtaaagtggatttagttttcgccccttcggtaaaagagatctacccgaacggtactgaaacccacacttacgttgacgttcctggcctttcgaccatgctggaaggtgccagccgtccgggacattttcgcggcgtttcgactattgtcagcaagctgttcaacctggtccagccggacatcgcctgcttcggtgaaaaagattttcagcaactggcgctgatccgcaaaatggttgccgatatgggcttcgatattgagattgtcggtgtgccaattatgcgcgccaaagacggtctggcgctaagttcccgtaacggttatctgacggcggaacaacgcaaaattgcgcctggtctgtacaaagttttaagttcgattgctgacaaattgcaggctggggaacgggatctcgatgaaattattaccattgcggggcaagaactgaatgaaaaaggcttccgcgccgatgatattcagattcgcgatgccgacacattgctggaagtttctgaaaccagcaaacgggcagtaattctggtagccgcctggcttggcgatgctcgcctgatcgacaacaaaatggtcgagctggcgtaatacttaactggcgctacggctgatggcgccagttattaatttaccccacgtcatctgtcataacacagg

SEQ ID NO: 19 - DNA, 1044 bp, (Artificial Sequence)
  source 1..1044: mol_type = genomic DNA
acatgcatgcttgacagctagctcagtcctaggtataatgctagcgttgcgggtgaggaggaacaatgaaaattaccgtattgggatgcggtgccttagggcaattatggcttacagcactttgcaaacagggtcatgaagttcagggctggctgcgcgtaccgcaaccttattgtagcgtgaatctggttgagacagatggttcgatatttaacgaatcgctgaccgccaacgatcccgattttctcgccaccagcgatctgctcctggtgacgctgaaagcatggcaggtttccgatgccgtcaaaagcctcgcgtccacactgcctgtaactacgccaatactgttaattcacaacggcatgggcaccatcgaagagttgcaaaacattcagcagccattactgatgggcaccaccacccatgcagcccgccgcgacggcaatgtcattattcatgtggcaaacggtatcacgcatattggcccggcacggcaacaggacggggattacagttatctggcggatattttgcaaaccgtgttgcctgacgttgcctggcataacaatattcgcgccgagctgtggcgcaagctggcagtcaactgcgtgattaatccactgactgccatctggaattgcccgaacggtgaattacgtcatcatccgcaagaaattatgcagatatgcgaagaagtcgcggcggtgatcgaacgcgaagggcatcatacttcagcagaagatttgcgtgattacgtgatgcaggtgattgatgccacagcggaaaatatctcgtcgatgttgcaggatatccgcgcgctgcgccacactgaaatcgactatatcaatggttttctcttacgccgcgcccgcgcgcatgggattgccgtaccggaaaacacccgcctgtttgaaatggtaaaaagaaaggagagtgaatatgagcgcatcggcactggtttgcctcgcccctggtagtgaagagactaattttcgaaaaaagacgctgaaaagcgtcttttttcgttttgggatctaaatcgag

SEQ ID NO: 20 - DNA, 1261 bp, (Artificial Sequence)
  source 1..1261: mol_type = genomic DNA
cggactggaagaagatctgtttgtctctgcgcgtccgaatattgaactgctgccggaaggccagtttaaataccacgtcgattttgagcatctgcatattggcgaagaaaccgggatgatttgcgtctcccggccgacgaatccaacaggcaatgtgattactgacgaagagttgctgaagcttgacgcgctggcgaatcaacacggcattccgctggtgattgataacgcttatggcgtcccgttcccgggtatcatcttcagtgaagcgcgcccgctatggaatccgaatatcgtgctgtgcatgagtctcaattccgacgtctaagaaaccattattatcatgacattaacctataaaaataggcgtatcacgaggccctttcgtcttcacctcgagtccctatcagtgatagagattgacatccctatcagtgatagagatactgagcacatcagcaggacgcactgaccgggcccaagttcacttaaaaaggagatcaacaatgaaagcaattttcgtactgaaacatcttaatcatgctaaggaggttttctaatgtatcgaacaatgatgagcggcaaacttcacagggcaactgttacggaagcaaacctgaactatgtgggaagcattacaattgatgaagatctcattgatgctgtgggaatgcttcctaatgaaaaagtacaaattgtgaataataataatggagcacgtcttgaaacgtatattattcctggtaaacggggaagcggcgtcatatgcttaaacggtgcagccgcacgccttgtgcaggaaggagataaggtcattattatttcctacaaaatgatgtctgatcaagaagcggcaagccatgagccgaaagtggctgttctgaatgatcaaaacaaaattgaacaaatgctggggaacgaaccagcccgtacaattttgtaaaagcctagcataaccccttggggcctctaaacgggtcttgaggggttttttgcatcaccaatatgaacggcattatcagcctggcacctggcggtattggtccggcgatgatgtgtgaaatgattaagcgtaacgatctgctgcgcctgtctgaaacagtcatcaaaccgttttactaccagcgtgttcaggaaactatcgccatcattcgccgctatttaccggaaaatcgctgcctgattcataaaccggaaggagccattttcctctggctatggtttaaggatttgcccattacgaccaagcagctctatcagc

SEQ ID NO: 21 - DNA, 1261 bp, (Artificial Sequence)
  source 1..1261: mol_type = genomic DNA
cggactggaagaagatctgtttgtctctgcgcgtccgaatattgaactgctgccggaaggccagtttaaataccacgtcgattttgagcatctgcatattggcgaagaaaccgggatgatttgcgtctcccggccgacgaatccaacaggcaatgtgattactgacgaagagttgctgaagcttgacgcgctggcgaatcaacacggcattccgctggtgattgataacgcttatggcgtcccgttcccgggtatcatcttcagtgaagcgcgcccgctatggaatccgaatatcgtgctgtgcatgagtctcaattccgacgtctaagaaaccattattatcatgacattaacctataaaaataggcgtatcacgaggccctttcgtcttcacctcgagtccctatcagtgatagagattgacatccctatcagtgatagagatactgagcacatcagcaggacgcactgaccgggcccaagttcacttaaaaaggagatcaacaatgaaagcaattttcgtactgaaacatcttaatcatgctaaggaggttttctaatgtaccgtacgttaatgagcgcaaaacttcacagagcgagagtgacggaagccaatttgaactacgtcggcagcgtgacaattgatgaagatttgctggatgctgtcggaatgatggcaaatgaaaaagtgcaaattgtgaataataataacggggcccggctggaaacgtacattattcccggtgaaaggggcagcggcgtcgtttgtttaaacggagctgccgcccgccttgtccaggttggagatgtcgtcatcatcgtgtcttatgcgatgatgtctgaagaggaagcaaagacccataagccgaaggttgccgttttgaacgagagaaacgaaatcgaggaaatgctgggtcaggagccagcccgtaccattctgtaaaagcctagcataaccccttggggcctctaaacgggtcttgaggggttttttgcatcaccaatatgaacggcattatcagcctggcacctggcggtattggtccggcgatgatgtgtgaaatgattaagcgtaacgatctgctgcgcctgtctgaaacagtcatcaaaccgttttactaccagcgtgttcaggaaactatcgccatcattcgccgctatttaccggaaaatcgctgcctgattcataaaccggaaggagccattttcctctggctatggtttaaggatttgcccattacgaccaagcagctctatcagc

SEQ ID NO: 22 - DNA, 1288 bp, (Artificial Sequence)
  source 1..1288: mol_type = genomic DNA
cggactggaagaagatctgtttgtctctgcgcgtccgaatattgaactgctgccggaaggccagtttaaataccacgtcgattttgagcatctgcatattggcgaagaaaccgggatgatttgcgtctcccggccgacgaatccaacaggcaatgtgattactgacgaagagttgctgaagcttgacgcgctggcgaatcaacacggcattccgctggtgattgataacgcttatggcgtcccgttcccgggtatcatcttcagtgaagcgcgcccgctatggaatccgaatatcgtgctgtgcatgagtctcaattccgacgtctaagaaaccattattatcatgacattaacctataaaaataggcgtatcacgaggccctttcgtcttcacctcgagtccctatcagtgatagagattgacatccctatcagtgatagagatactgagcacatcagcaggacgcactgaccgggcccaagttcacttaaaaaggagatcaacaatgaaagcaattttcgtactgaaacatcttaatcatgctaaggaggttttctaatgctgcgcaccatcctcggaagtaagattcaccgagccactgtcactcaagctgatctagattatgttggctctgtaaccatcgacgccgacctggttcacgccgccggattgatcgaaggcgaaaaagttgccatcgtagacatcaccaacggcgctcgtctggaaacttatgtcattgtgggcgacgccggaacgggcaatatttgcatcaatggtgccgctgcacaccttattaatcctggcgatcttgtgatcatcatgagctaccttcaggcaactgatgcggaagccaaggcgtatgagccaaagattgtgcacgtggacgccgacaaccgcatcgttgcgctcggcaacgatcttgcggaagcactacctggatccgggcttttgacgtcgagaagcatttaaaagcctagcataaccccttggggcctctaaacgggtcttgaggggttttttgcatcaccaatatgaacggcattatcagcctggcacctggcggtattggtccggcgatgatgtgtgaaatgattaagcgtaacgatctgctgcgcctgtctgaaacagtcatcaaaccgttttactaccagcgtgttcaggaaactatcgccatcattcgccgctatttaccggaaaatcgctgcctgattcataaaccggaaggagccattttcctctggctatggtttaaggatttgcccattacgaccaagcagctctatcagc

SEQ ID NO: 23 - DNA, 2629 bp, (Artificial Sequence)
  source 1..2629: mol_type = genomic DNA
ggcagaaaatcagccagttccgcgcccgccatcccgcaattggcgcgggcaaacaaacgacacttttgctgaagcagggctacggctttgttcgtgagcatggcgacgataaagtgctggtcgtctgggcagggcaacagtaacttttccggcttcccgttcgtcagtacctcgggaagccgccaaccaggataaaatgtcagccctaatcagcgttgcaggataaagcaccgctcactcttcaacagaccgatttgcaccccagcaaatgtagcgttattgttaccttccttgctacagagttcttgacaattaatcatccggctcgtataatgtgtggacaagattcaggacggggaactaactatgaatggcgcacagtgggtggtacatgcgttgcgggcacagggtgtgaacaccgttttcggttatccgggtggcgcaattatgccggtttacgatgcattgtatgacggcggcgtggagcacttgctatgccgacatgagcagggtgcggcaatggcggctatcggttatgctcgtgctaccggcaaaactggcgtatgtatcgccacgtctggtccgggcgcaaccaacctgataaccgggcttgcggacgcactgttagattccatccctgttgttgccatcaccggtcaagtgtccgcaccgtttatcggcactgacgcatttcaggaagtggatgtcctgggattgtcgttagcctgtaccaagcacagctttctggtgcagtcgctggaagagttgccgcgcatcatggctgaagcattcgacgttgcctgctcaggtcgtcctggtccggttctggtcgatatcccaaaagatatccagttagccagcggtgacctggaaccgtggttcaccaccgttgaaaacgaagtgactttcccacatgccgaagttgagcaagcgcgccagatgctggcaaaagcgcaaaaaccgatgctgtacgttggcggtggcgtgggtatggcgcaggcagttccggctttgcgtgaatttctcgctgccacaaaaatgcctgccacctgtacgctgaaagggctgggcgcagtagaagcagattatccgtactatctgggcatgctgggaatgcatggcaccaaagcggcgaacttcgcggtgcaggagtgcgacttgctgatcgccgtgggtgcacgttttgatgaccgggtgaccggcaaactgaacaccttcgcaccacacgccagtgttatccatatggatatcgacccggcagaaatgaacaagctgcgtcaggcacatgtggcattacaaggtgatttaaatgctctgttaccagcattacagcagccgttaaatatcaatgactggcagctacactgcgcgcagctgcgtgatgaacatgcctggcgttacgaccatcccggtgacgctatctacgcgccgttgttgttaaaacaactgtcagatcgtaaacctgcggattgcgtcgtgaccacagatgtggggcagcaccagatgtgggctgcgcagcacatcgcccacactcgcccggaaaatttcatcacctccagcggcttaggcaccatgggttttggtttaccggcggcggttggcgcgcaagtcgcgcgaccaaacgataccgtcgtctgtatctccggtgacggctctttcatgatgaatgtgcaagagctgggcaccgtaaaacgcaagcagttaccgttgaaaatcgtcttactcgataaccaacggttagggatggttcgacaatggcagcaactgtttttccaggaacgatatagcgaaaccacccttaccgataaccccgatttcctcatgttagccagcgccttcggcatccctggccaacacatcacccgtaaagaccaggttgaagcggcactcgacaccatgctgaacagtgatgggccatacctgcttcatgtctcaatcgacgaacttgagaacgtctggccgctggtgccgcctggtgccagtaattcagaaatgttggagaaattatcatgatgcaacatcaggtcaatgtatcggctcgcttcaatccagaaaccttagaacgtgttttacgcgtggtgcgtcatcgtggtttccacgtctgctcaatgaatatggccgccgccagcgatgcacaaaatataaatatcgaattgaccgttgccagcccacggtcggtcgacttactgtttagtcagttaaataaactggtggacgtcgcacacgttgccatctgccagagcacaaccacatcacaacaaatccgcgcctgagcgcaaaaggaatataccagaaaagagacgcttttagagcgtcttttttcgttttggagctactcacactgcttgccggaatgctgcgcgagaagttgggttgggatatcgaaccacagaatattgcactaacaaacggcagccagagcgcgtttttctacttatttaacctgtttgccggacgccgtgccgatggtcgggtcaaaaaagtgctgttcccgcttgcaccggaatacattggctatgctgacgccggactggaagaagatctgtttgtctctgcgcgtccgaatattgaactgctgccggaaggccagtttaaataccacgtcgattttgagcatctgcatattggc

SEQ ID NO: 24 - DNA, 63 bp, (Artificial Sequence)
  source 1..63: mol_type = genomic DNA
cgcggatcccaattaatcatccggctcgtataatgtgtggagcacaacatcaatttatcagga

SEQ ID NO: 25 - DNA, 30 bp, (Artificial Sequence)
  source 1..30: mol_type = genomic DNA
acatgcatgccctgtgttatgacagatgac

SEQ ID NO: 26 - DNA, 65 bp, (Artificial Sequence)
  source 1..65: mol_type = genomic DNA
acatgcatgcttgacagctagctcagtcctaggtataatgctagcgttgcgggtgaggaggaaca

SEQ ID NO: 27 - DNA, 90 bp, (Artificial Sequence)
  source 1..90: mol_type = genomic DNA
ctcgatttagatcccaaaacgaaaaaagacgcgcttttcagcgtcttttttcgaaaattagtctcttcactaccagggatgactatcgag

SEQ ID NO: 28 - DNA, 30 bp, (Artificial Sequence)
  source 1..30: mol_type = genomic DNA
tgggtctaccgttttagagctagaaatagc

SEQ ID NO: 29 - DNA, 29 bp, (Artificial Sequence)
  source 1..29: mol_type = genomic DNA
gcttggaaaggactagtattatacctagg

SEQ ID NO: 30 - DNA, 19 bp, (Artificial Sequence)
  source 1..19: mol_type = genomic DNA
cggactggaagaagatctg

SEQ ID NO: 31 - DNA, 39 bp, (Artificial Sequence)
  source 1..39: mol_type = genomic DNA
tttcttagacgtcggaattgagactcatgcacagcacga

SEQ ID NO: 32 - DNA, 40 bp, (Artificial Sequence)
  source 1..40: mol_type = genomic DNA
tcgtgctgtgcatgagtctcaattccgacgtctaagaaac

SEQ ID NO: 33 - DNA, 44 bp, (Artificial Sequence)
  source 1..44: mol_type = genomic DNA
gatctcctttttaagtgaacttggggtcagtgcgtcctgctgat

SEQ ID NO: 34 - DNA, 44 bp, (Artificial Sequence)
  source 1..44: mol_type = genomic DNA
atcagcaggacgcactgaccccaagttcacttaaaaaggagatc

SEQ ID NO: 35 - DNA, 39 bp, (Artificial Sequence)
  source 1..39: mol_type = genomic DNA
tgccgttcatattggtgatgcaaaaaacccctcaagacc

SEQ ID NO: 36 - DNA, 39 bp, (Artificial Sequence)
  source 1..39: mol_type = genomic DNA
ggtcttgaggggttttttgcatcaccaatatgaacggca

SEQ ID NO: 37 - DNA, 19 bp, (Artificial Sequence)
  source 1..19: mol_type = genomic DNA
gctgatagagctgcttggt

SEQ ID NO: 38 - DNA, 20 bp, (Artificial Sequence)
  source 1..20: mol_type = genomic DNA
ggagctactcacactgcttg

SEQ ID NO: 39 - DNA, 20 bp, (Artificial Sequence)
  source 1..20: mol_type = genomic DNA
cgcatacattgatgcgtatg

SEQ ID NO: 40 - DNA, 30 bp, (Artificial Sequence)
  source 1..30: mol_type = genomic DNA
acggtccacagttttagagctagaaatagc

SEQ ID NO: 41 - DNA, 29 bp, (Artificial Sequence)
  source 1..29: mol_type = genomic DNA
cgtagttacagactagtattatacctagg

SEQ ID NO: 42 - DNA, 20 bp, (Artificial Sequence)
  source 1..20: mol_type = genomic DNA
ggcagaaaatcagccagttc

SEQ ID NO: 43 - DNA, 56 bp, (Artificial Sequence)
  source 1..56: mol_type = genomic DNA
tccacacattatacgagccggatgattaattgtcaagaactctgtagcaaggaagg

SEQ ID NO: 44 - DNA, 56 bp, (Artificial Sequence)
  source 1..56: mol_type = genomic DNA
ttgacaattaatcatccggctcgtataatgtgtggacaagattcaggacggggaac

SEQ ID NO: 45 - DNA, 55 bp, (Artificial Sequence)
  source 1..55: mol_type = genomic DNA
cgaaaaaagacgctctaaaagcgtctcttttctggtatattccttttgcgctcag

SEQ ID NO: 46 - DNA, 58 bp, (Artificial Sequence)
  source 1..58: mol_type = genomic DNA
cagaaaagagacgcttttagagcgtcttttttcgttttggagctactcacactgcttg

SEQ ID NO: 47 - DNA, 38 bp, (Artificial Sequence)
  source 1..38: mol_type = genomic DNA
gccaatatgcagatgctcatgagcatctgcatattggc

SEQ ID NO: 48 - DNA, 19 bp, (Artificial Sequence)
  source 1..19: mol_type = genomic DNA
cacgttcggatatgaactg

SEQ ID NO: 49 - DNA, 19 bp, (Artificial Sequence)
  source 1..19: mol_type = genomic DNA
cgtcaagcttcagcaactc